European Patent Application EP 4 741 505 A1, published May 13, 2026. Title: 一种谷氨酸棒杆菌中的非编码sRNA及其应用. Applicant: 大连医诺生物股份有限公司. Application WO. The sequence listing filed with the application follows.

SEQUENCE LISTING (6 sequences)

SEQ ID NO: 1 - DNA, 115 bp, synthetic construct
  source 1..115: mol_type = other DNA
tgcttcattgttagacaattctctcttttttcattaaggacaaaaatgaatcgagaaaaccattacccgaaaagttttaaagttttttgggcttggatttttattccactctttg

SEQ ID NO: 2 - DNA, 115 bp, synthetic construct
  source 1..115: mol_type = other DNA
tcgttgagaagtaatcaattctgacttttttcattaaggacaaaaatgaatgcagaaaaccattacccgaaaagttttaaagttttttgggcttggatttttattccactctttg

SEQ ID NO: 3 - DNA, 21 bp, synthetic construct
  source 1..21: mol_type = other DNA
ggctgttttggcggatgagag

SEQ ID NO: 4 - DNA, 23 bp, synthetic construct
  source 1..23: mol_type = other DNA
ttgttatccgctcacaattccac

SEQ ID NO: 5 - DNA, 23 bp, synthetic construct
  source 1..23: mol_type = other DNA
gtggaattgtgagcggataacaa

SEQ ID NO: 6 - DNA, 21 bp, synthetic construct
  source 1..21: mol_type = other DNA
ctctcatccgccaaaacagcc